European Patent Application EP 4 124 855 A1, published February 1, 2023. Title: Biosensor for the detection of hepatitis C virus. Applicant: International Iberian Nanotechnology Laboratory (INL) Consejo Superior de Investigaciones Cientificas (CSIC) Instituto Nacional de Técnica Aeroespacial (INTA) UNIVERSIDADE DO MINHO. The sequence listing filed with the application follows.

SEQUENCE LISTING (3 sequences)

SEQ ID NO: 1 - DNA, 76 bp, Artificial Sequence
  5´-3´sequence of the Apt-HCVcore_01
gcggatccagactggtgtgccgtatccctcccttgtaattatttgttccatccgttccgccctaaagacaagcttc

SEQ ID NO: 2 - DNA, 76 bp, Artificial Sequence
  5´-3´ complementary reverse sequence of the Apt-HCVcore_01
gaagcttgtctttagggcggaacggatggaacaaataattacaagggagggatacggcacaccagtctggatccgc

SEQ ID NO: 3 - DNA, 76 bp, Artificial Sequence
  D-ACTG
gcggatccagactggtgtactgactgactgactgactgactgactgactgactgactggccctaaagacaagcttc